European Patent Specification EP 3 711 057 B1, published July 17, 2024. Title: METHOD, DEVICE, AND COMPUTER PROGRAM FOR GENERATING PROTEIN SEQUENCES WITH AUTOREGRESSIVE NEURAL NETWORKS. Applicant: INSTITUT PASTEUR. The sequence listing filed with the application follows.

SEQUENCE LISTING (77 sequences)

SEQ ID NO: 1 - protein, 337 aa, Kineococcus radiotolerans
MVDTHGQPLKLGYKASAEQFAPGKLADFAVQAEEQGLDSVWISDHFQPWRHVDGHAPSALVWLPWVAAKTSRVQLGTSVLTPTLRYNPAVIAQAFATLGCLAPGRAILGIGTGEALNETAVGVTFPETRERFARLREAVRLIKQLWSEERVTFEGEYYNLHDATVYDRPEQPVPIYVAAGGPGVTKYAGRAGDGYICTSGKGMDLYSETLLPALREGLEASGRTEGQIDRTIEIKLSFDEDPAQALENTRFWAPLSLTAEQKSSVHDPIEMARLADELPIEQVAKRWIVSSDPTEVAAAVQGYVDAGFTHLVFHAPGQDQSRFLTQFSADVVPLLRP

SEQ ID NO: 2 - protein, 340 aa, Artificial Sequence
  reconstructed sequence
MSDTFGASLSEYGSAAQFAPAAPGDLWNAVARAAEAGGFDMFWADHHHPDGGQLPAGEGLMTVAAAAATATRKLTLGLVASTNRVRQVLALARAAEVLSVLSSGRVLLGLGTGGHDRVVAAYGVPYPDRERYRRLRESLRIFRELWSGETVSFEGEYYRTHDVYGYDIPAGGPVPIIVAGGAPAERYRGAAGHDFLCVSGSWAEAYREKLLPAVDAGADAAGRDDAFRRRVIELKSYFDADEAAALREETFWAPLSLTAAAEHDVLDAVAEPLGADELVREQVAKRWIVGSSPDDIAALIDPHVDAGLNYLLFHAPGQDQDRFLDLFGELVEERLRAVAG

SEQ ID NO: 3 - protein, 340 aa, Artificial Sequence
  reconstructed sequence
MSDAFGGTLSENGFFAPFAPAGPDALYELAERAGLAENGFQDWWFPHPHLDGTPTWPEADYWLAWATAVTSRLRLGTWVLSNTFRHPVVLAKSFATIDQLSNGRVLLGLGSGGVDRLEGAVEGEYPERVERFERSAESIRIFREMWSGDTVSFDGEYYTTHDVYFYERPEQPPPVYIAAGGPGVAKYNGRAGDGFLCTSGKWMDANREKLLPAFKEGAARTGRDADEIRRHIEIDLSYDEDYEAALDGWTPWAPLSLTAEQPVAVTDPLAVPGADDLLPREVIASRWIVGSSPDEVAALIQPHVDAGLNYLMFHVPGGDQDRFLELFEQAVEELGRTGFG

SEQ ID NO: 4 - protein, 340 aa, Artificial Sequence
  reconstructed sequence
MSDTSRGILGYKGYLAQFAPADPPALWVAAVAEEAGRRTFMFWDHHWYPAGGTPGFTEGWMWLAAAAARTSRIRLGTLVYSTPFRHPAVVAKSFATVDHISGGRVLLGLGAGSGHDEIAAYGFEWPDAGERYARLEESVRIIKELWSGETVSFDGEYYRTHDALVYPRPAQGPPVYIAAGGPAVAKRAGRVGDGFICTSLGGNDLLRESLEALRAGYEKAGRDGDFVRKRVLELKDSYDLAERAALALTAFWAPLGLTPAQKHLVLDPAPMPERADELVKEFVASRWIVGSSPEEIAALIEPHVDAGLFHLVFHAPGGDQDRFLDLFGRDVEPLLRSPAA

SEQ ID NO: 5 - protein, 338 aa, Artificial Sequence
  reconstructed sequence
MSDTGTATLSEGGTAEQFSPEAPFDLCGTAAEAGFLADHFGFWDHYWSPSEKKLDWSGALWTAVAAATTTTRLARGVLVVSPLSNHKVALARQATTVAQVSGNRVLLGLGSGGHNRIEAAVEGDYPEARERYAQLRESIRIIRELWSGETVSFEGEYYSTHDVYRYERPAQGPPVYIAAGSPRVARYAGRAGDNFLCTSGHTMDAYREKLLPLWKGGDAAGKDPDDLRARVDIQILSYTNDEEAAAELTRGWAPLGLYRAAKHDVLDPVPLPQDADELVRELVASRWVVGSSPEDVAALIGPQVDAGLNYGLFFVPGVDQSFDLSLGLALNAELLRSL

SEQ ID NO: 6 - protein, 339 aa, Artificial Sequence
  reconstructed sequence
MSDTPSGKLLDYGTGAQFAPDGPERFASMADAAGLAERTFSDWDHFGYPDKGGAGWTPAWGWLAALIARTSRIKLGTAVTSVNFRHPVVAAKSAATVDIISQGRADLGLGAGAIDEIEAAVEGAWPPAKERYERLREYLEIIRELWTGETVSFEGKYYETHGAQFYDRPDQPVPPYIAAGGPTVAKYAGAAGDGFLCVSGKGMDLYDEKLLPGFKEGIDALGRDFDRIGRTIEFKLSFDEDYEAALDLTRGWAPLSLTAEQNFDVAGPIAMPQDADELVRELFAKRWIAGNPEENAVELIQLQVGAGLDYGMFHVPVGDQDRFEELFDRFAEQLRRLGA

SEQ ID NO: 7 - protein, 337 aa, Artificial Sequence
  reconstructed sequence
MSDTAGGALGYPGALAQFSPADPDALRIVAEAAGYAEDAFQDWTFPWHPLPGQPGWSPAWYILGAATARTSRLALSTLVTSVNFRRPAVLAKSFATVDHLSNGRVLLGLGSGSAERLEAAVEGEWPEKRERFERLEESVTLIRELWSGETVSFDGEHYTTHDAYGYPMPAQGPVPVLVTGGAPVAKVAGRAGDGYLCVSGKGPTDREWKLLPAVREGAAAAGRDADEIKRTIEIKLSFDDDVAAALREERVWAGLALTAAQKHSVWDPVAAPDDADELIRELVAKLVIVGSPEEVAAELVKWGEAWGLDYALFHLPGGDQDRLLELFGERVEALGRA

SEQ ID NO: 8 - protein, 339 aa, Artificial Sequence
  reconstructed sequence
MTFTFGGPLADKGSGPQFAPAAEVLDDYVALAEAAERAGFNLWTPYWHPLENTGPFPEWWMWLLGAAATTSRLRLGTLVLSPTFNNPVRVAEQFATVDQLSGGRLDLGLGAGSGHNEYAAFGFDYPEKKERFARLAESVRIFREEWTGTTKSFSGEYYTVNDAYFYPRPEQPPVPLIAAGGPTVAKRAGRIGDGFLCTSGKGMDEYREKLLTAHAEAGAAGQRPDALRRRVGIKLNPYEVDEKAALEETGIDAWLPLFADQKPSVVGPREMPVDARDLPRREALRRWIASSTPDLIAELIKPHVDAGLFHLVFAAPGHDQDRFLELFDEDVAQYARSLG

SEQ ID NO: 9 - protein, 339 aa, Artificial Sequence
  reconstructed sequence
MTDTSPATLSEIGTSAQFAPADLVDLVVAAEQAGFAGVGFSDWDHFWSPLEGKGTWSEAMGWLAALSRTAGRKALGTLVLSNSFRPQVVFARHATTVALLSGRRVLLGLGAGGVDRLAGGVEGDWPEPRERYERLRESVEIIRRLWTGETVSFDGEYYRTHDAYGYPVSEQGPVPIIVAGSPEVAKRAARVGDGFLCFSGSGPDAYDESLLPAFKAGAAAGGRDDAFRDRVIELKSYYDVAERAALEETRGWAPLSLARDQKHSVADPVAMPGRDDELVKEQVAKRWIVGSSPDEAVAAIQPYVDAGLFHLVFHAPGGDQDRFLELFDEDVRAYLRSLA

SEQ ID NO: 10 - protein, 367 aa, Yersinia enterocolitica
MKIGVFIPIGNNGWLISSNAPQYMPSFELNKAIVQQAEHYQFDFALSMIKLRGFGGKTEFWDHNLESFTLMAGLAAVTSRIKIYATAATLTLPPAIVARMASTIDSISNGRFGLNVVTGWQKPEYEQMGLWPGDEYFSRRYDYLSEYVEVLQDFWGTGQSDFNGEFFQMDDCRVSPQPQTPIKLICAAQSDAGMAFSAKYADYNFCFGKGVNTPTAFAPTAARLQKAAEQAGREVSSYVLFMIIADETDELARAKWESYKAGADTEALAWLTEQSGKDTQSGADTNVRQMADPTSAVNINMGTLVGSYANVAKMMDDIATVPGTEGILLTFDDFLSGIENFGQHIQPLMNSRADIVDTLPPAAREVA

SEQ ID NO: 11 - protein, 367 aa, Artificial Sequence
  reconstructed sequence
MKIGVFIPIGNNGWLISTNAPQYMPSFELNKAIVQKAEHYQFDFALSMIKLRGFGGKTEFWDHNLESFTLMAGLAAVTSRIKIYATAATLTLPPAIVARMASTIDSISNGRFGLNVVTGWQKPEYEQMGLWPGDEYFSRRYDYLSEYVQVLRDLWGTGKSDFKGEFFQMDDCRVSPQPQAPIKVICAGQSDAGMAFSAKYADYNFCFGKGVNTPTAFAPTAARMKEAAEKAGRDVSSYVLFMIIADETDEAARAKWESYKAGADTEALAWLTEQSGKDTKSGADTNVRQMADPTSAVNINMGTLVGSYANVARMMDEIATVPGTEGILLTFDDFLSGIENFGQRIQPLMKSRADIIPTTPEAAREVA

SEQ ID NO: 12 - protein, 393 aa, Artificial Sequence
  generated sequence
MPVSWLLLGHSSGVGLGGPDAAAAAEGAYGFRAAVVAERVGFDGVLLGARGSPEYPATVARLLAEAALHQLRLGAGVTATSTYAPAAGVEVLGTLASLFPRDIILGLGISTGARHDEAGGRDHFQRWEGDFGDHYPAVRGALGLWTDEEVLREASFASPYYPRGVEGWRVVVSPRPPRAGLWLGEKPEDVGVLGDDVALLHAFRPVFGRSGPAVAGLLGADVPAWAPAGLHPIVDVRLIWGGSPSDAQFLADLERAEALAFARAEGMRGVEAEPTRRLLAEATSGAPDEAAAGTLAAQQVDVEIDGTPWWAETPRTVSAGLGAAELGTRLVAVGLDAVATGATSVDGWSTVGGLAGGGDGFWIGPELYADGARRGAAFDGDVASLSPGRVADH

SEQ ID NO: 13 - protein, 339 aa, Streptomyces sp. AA4
MDTRTSGITIGYKASAEQFGPRHLVELAVLAERRGFDSVLVSDHYQPWRHRNGHAPFSMAWLAAAGERTERVRLGTSVLTATFRYHPAVVAQAFGTLGALCPGRVMLGLGTGEALNEVAVARMEWPGFEERFARLREAIDLIRRLWTEERVSFDGEYYRTENATVYDRPSRPVPVYVAAGGPVVAKYAGRIADGFICTSGKGMELYTEKLQPAVDAGAEAGREPADVARTIEIKLSYDTDAEAAAENTRFWAPLSLTADQKHGVSDPLAMERAADELPMSQIASRWIVSSDPDEVVERIRPYVDAGFTDLVLHAPGHDQARFLELARQDLLPRLRNLGG

SEQ ID NO: 14 - DNA, 53 bp, Artificial Sequence
  Primer
taatataatagcgaacgttgagtactaaagtttccaaatttcatagagagtcc

SEQ ID NO: 15 - DNA, 53 bp, Artificial Sequence
  Primer
ctatgaaatttggaaactttagtactcaacgttcgctattatattagctaagg

SEQ ID NO: 16 - DNA, 20 bp, Artificial Sequence
  Primer
tcatttcgaaccccagagtc

SEQ ID NO: 17 - DNA, 20 bp, Artificial Sequence
  Primer
cgccttcttgacgagttctt

SEQ ID NO: 18 - DNA, 40 bp, Artificial Sequence
  Primer
tctatcaacaggagtccaagcgagctcgatatcaaattac

SEQ ID NO: 19 - DNA, 41 bp, Artificial Sequence
  Primer
ttttgaattcgacgtcgacgtcgatatctggcgaaaatgag

SEQ ID NO: 20 - DNA, 40 bp, Artificial Sequence
  Primer
atcgagctcgcttggactcctgttgatagatccagtaatg

SEQ ID NO: 21 - DNA, 40 bp, Artificial Sequence
  Primer
ccagatatcgacgtcgacgtcgaattcaaaagatcttaag

SEQ ID NO: 22 - DNA, 42 bp, Artificial Sequence
  Primer
cacaggagactttctaatgaaatttggaaactttttgcttac

SEQ ID NO: 23 - DNA, 39 bp, Artificial Sequence
  Primer
ctcgacaaccgatccctaatataatagcgaacgttgttt

SEQ ID NO: 24 - DNA, 41 bp, Artificial Sequence
  Primer
gtttccaaatttcattagaaagtctcctgtgcatgattaag

SEQ ID NO: 25 - DNA, 38 bp, Artificial Sequence
  Primer
tcgctattatattagggatcggttgtcgagtaaggatc

SEQ ID NO: 26 - DNA, 29 bp, Artificial Sequence
  Primer
cattagaaagtctcctgtgcatgattaag

SEQ ID NO: 27 - DNA, 23 bp, Artificial Sequence
  Primer
ggatcggttgtcgagtaaggatc

SEQ ID NO: 28 - DNA, 33 bp, Artificial Sequence
  Primer
caattttcgtactgaaacatcttaatcatgcac

SEQ ID NO: 29 - DNA, 25 bp, Artificial Sequence
  Primer
cgttttatttgatgcctggagatcc

SEQ ID NO: 30 - protein, 360 aa, Artificial Sequence
  reconstructed sequence
MKFGNFLLTYQPPQFSQTEVMKRLVKLGRVSEECGFDTVWLLEHHFTEFGLLGNPYVAAAYLLGATKKLNVGTAAIVLPTAHPVRQLEDVNLLDQMSKGRFRFGICRGLYNKDFRVFGVDMNNTRALMECWYGLIKNGMTEGYVEADNEHIKFHKVKVNPTAYSQGGAPVYVVAESASTTEWAAQHGLPMILSWIINTNEKKAQLELYNEVAQEYGHDVHNIDHCLSYITSVDHDSIKAKEICRNFLGHWYDSYVNATTIFDDSDQTKGYDFNKGQWRDFVLKGHKDTNRRIDYSYEINPVGTPKECIDIIQTDIDATGISNICCGFEANGTVDEIIASMKLFQSDVMPFLKEKQRSLLY

SEQ ID NO: 31 - protein, 359 aa, Artificial Sequence
  reconstructed sequence
MKFGNFLLTYQPPQFSQTEVMQRLVNLGRASEECGFDTVWLLEHHFTEFGLLGNPYVAAAYLLGATKHLNVGTAAIVLPTAHPVRQLEDVNLLDQMSKGRFRFGICRGLYNKDFNVFGVDMNNTRALTECWYGLIKNGMTEGYMEADNEHIKFHKVKVNPTAYSKGGAPVYVVAESASTTEWAAQHGLPMILSWIINTNEKKAQIDLYNEVAQEHGHDVHNIDHCLSYITSVDHDSKKAKEICRDFLGHWYDSYVNATTIFDDSDQTKGYGFNKGQWHDFVLKGHKDTNRRVDYSYEINPVGTPQECIDIIQTDIDATGISNICCGFEANGTVDEIIASMKLFQSDVMPFLKEKQRSLL

SEQ ID NO: 32 - protein, 359 aa, Artificial Sequence
  reconstructed sequence
MKFGNFLLTYQPPQFSQTEVMQRLVKLGRVSEECGFDTVWLLEHHFTEFGLLGNPYVAAAYLLGATKKLNVGTAAIVLPTAHPVRQLEDVNLLDQMSKGRFRFGICRGLYNKDFRVFGVDMNNTRALMECWYGLIKNGMTEGYMEADNEHIKFHKVKVNPTAYTQGGAPIYVVAESASTTEWAAQFGLPMILSWIINTNEKIAQLELYNEVAQEYGHDVHNIDHCLSYITSVDHDSIKAKEICRQFLGHWYDSYVNATTIFDDSDQTKGYDFNKGQWRDFVLKGHKDTNRRIDYSYEINPVGTPKECIDIIQTDIDATGISNICCGFEANGTVDEIIASMKLFQSDVMPFLKEKQRSLL

SEQ ID NO: 33 - protein, 359 aa, Artificial Sequence
  reconstructed sequence
MKFGNFLLTYQPPQFSQTEVMQRLVKLGRVSEECGFDTVWLLEHHFTEFGLLGNPYVAAAYLLGATKKLNVGTAAIVLPTAHPVRQLEDVNLLDQMSKGRFRFGICRGLYNKDFRVFGVDMNNTRALMECWYGLIKNGMTEGYVEADNEHIKFHKVKVNPTAYSQGGAPVYVVAESASTTEWAAQHGLPMILSWIINTNEKIAQIELYNEVAQEYGHDIHNIDHCLSYITSVDHDSIKAKEICRNFLGHWYDSYVNATTIFDDSDKTKGYGFNKGQWRDFVLKGHKDTNRRIDYSYEINPVGTPKECIDIIQTDIDATGISNICCGFEANGTVDEIIASMKLFQSDVMPFLKETQRSLL

SEQ ID NO: 34 - protein, 360 aa, Artificial Sequence
  reconstructed sequence
MKFGNFLLTYQPPQLDQSEVMARLVKLGRVSEECGFDTVWLLEHHFTEFGLLGNPYVAAAYLLGATKKLNVGTAAIVLPTAHPVRQLEDVNLLDQMSKGRFRFGICRGLYNKDFRVFGVDMNNSRALMECWYDLIKEGMTEGYVEADTEHIKFHKVKHLPTAYSQGGAPVYVVAESASTTEWAAQHGLPMILSWIINTNEKKAQLELYNEVAQEYGHDIHNIDHCLSYITSVDHDSIRAKEKCVNHLGHWYDSYVNATTIFDDSDQTKGYGFNKGQWRDFVLKGHKDTNRRIDYSYEINPVGTPNECIDIIQTDIDATGISNICCGFEANGTVDERIASMLLFQSDVMPFLKEKQRSLLY

SEQ ID NO: 35 - protein, 360 aa, Artificial Sequence
  reconstructed sequence
MKFGNFLLTYQPPQFSQTEVMQRLVKLGRVSEECGFDTVWLLEHHFTEFGLLGNPYVAAAYLLGATKKLNVGTAAIVLPTAHPVRQLEDVNLLDQMSKGRFRFGICRGLYNKDFRVFGVDMNNTRALMECWYGLIKNGMTEGYVEADNEHIKFHKVKVNPTAYSQGGAPVYVVAESASTTEWAAQFGLPMILSWIINTNEKKAQLELYNEVAQEYGHDIHNIDHCLSYITSVDHDSIKAKEICRNFLGHWYDSYVNATTIFDDSDQTKGYGFNKGQWRDFVLKGHKNTNRRIDYSYEINPVGTPKECIDIIQTDIDATGISNICCGFEANGTVDEIIASMKLFQSDVMPFLKEKQRSLLY

SEQ ID NO: 36 - protein, 359 aa, Artificial Sequence
  reconstructed sequence
MKFGNFLLTYQPPQFSQTEVMKRLVKLGRVSEECGFDTVWLLEHHFTEFGLLGNPYVAAAYLLGATKKLNVGTAAIVLPTAHPVRQLEDVNLLDQMSKGRFRFGICRGLYNKDFRVFGVDMDNTRALMECWYGLIKNGMTEGYVEADNEHIKFHKVKVNPTAYSQGGAPIYVVAESASTTEWAAQHGLPMILSWIINTNEKKAQLELYNEVAQEHGHDVHNIDHCLSYITSVDHDSIKAKEICRNFLGHWYDSYVNATTIFDDSDQTKGYGFNKGQWRDFVLKGHKDTNRRIDYSYEINPVGTPKECIDIIQTDIDATGISNICCGFEANGTVDEIIASMKLFQSDVMPFLKEKQRSLL

SEQ ID NO: 37 - protein, 360 aa, Artificial Sequence
  reconstructed sequence
MKFGNFLLTYQPPQFSQTEVMQRLVKLGRVSEECGFDTVWLLEHHFTEFGLLGNPYVAAAYLLGATKKLNVGTAAIVLPTAHPVRQLEDVNLLDQMSKGRFRFGICRGLYNKDFRVFGVDMNNTRALMECWYGLIKNGMTEGYMEADNEHIKFHKVKVNPTAYSQGGAPVYVVAESASTTEWAAQHGLPMILSWIINTNEKKAQLELYNEVAQEHGHDIHNIDHCLSYITSVDHDSIKAKEICRNFLGHWYDSYVNATTIFDDSDQTKGYDFNKGQWRDFVLKGHKDTNRRIDYSYEINPVGTPKECIDIIQTDIDATGISNICCGFEANGTVDEIIASMKLFQSDVMPFLKEKQRSLLY

SEQ ID NO: 38 - protein, 360 aa, Artificial Sequence
  reconstructed sequence
MKFGNFLLTYQPPQLPQTEVMKRLVKLGRVSEGCGFDTVWLLEHHFTEFGLLGNPYVAAAHLLGATKKLNVGTAAIVLPTAHPIRQLEDVNLLDQMSKGRFRFGICRGLYNKDFRVFGTDMNNSRVLMECWYGLIKNGMTEGYMEADNEHIKFHKVKVNPTAYSRGGAPVYVVAESASTTEWAAQFGLPMILSWIINTNEKKAQAELYNEVALEYGRDIHNIDHCLSYITSVDHDSIKAKEICRNFLGHWYDSYVNATTIFDDSDQTKGYDFNKGQWRDFVLKGHKDTNRRIDYSYEINPVGTPEECIDIIQTDIDATGISNICCGFEANGTVDEIIASMKLFQSDVMPFLKEKQRSLLY

SEQ ID NO: 39 - protein, 360 aa, Artificial Sequence
  reconstructed sequence
MKFGNFLLTYQPPQFSQTEVMKRLVKLGRVSEECGFDTVWLLEHHFTEFGLLGNPYVAAAYLLGATKKLNVGTAAIVLPTAHPVRQLEDVNLLDQMSKGRFRFGICRGLYNKDFRVFGVDMNNSRALMECWYGLIKNGMTEGYVEADNEHIKFHKVKVNPTAYSQGGAPIYVVAESASTTEWAAQHGLPMILSWIINTNEKKAQLEFYNEVAQEYGHDIHNIDHCLSYITSVDHDSIKAKEICRNFLGHWYDSYVNATTIFDDSDQTKGYGFNKGQWRDFVLKGHKNTNRRIDYSYEINPVGTPKECIDIIQTDIDATGISNICCGFEANGTVDEIIASMKLFQSDVMPFLKEKQRSLLY

SEQ ID NO: 40 - protein, 360 aa, Artificial Sequence
  reconstructed sequence
MKFGNFLLTYQPPEFSQTEVMKRLVKLGRVSEECGFDEVWLLEHHFTEFGLLGNPYVAAAHLLGATKKLNVGTAAIVLPTAHPVRQLEDVNLLDQMSKGRFRFGICRGLYNKDFRVFGVDMNNSRVLMECWYGLMKNGMTEGYMEADNEHIKFHKVKVNPTAYTQGGAPIYVVAESASTTEWAAQHGLPMILSWIINNNEKIYQAKFYNEVAQESGHDIHNIDHCLSYITSVDHDSIKAKEICRNFLGHWYDSYVNATTIFDDSDKTKGYDFNKGQWRDFVLKGHKDTNRRIDYSYEINPVGTPKECIDIIQTDIDATGISINCCGFEANGTVDEIIASMKLFQSDVMPFLKEKQRSLLY

SEQ ID NO: 41 - protein, 360 aa, Artificial Sequence
  reconstructed sequence
MKFGNFLLTYQPPQFSQTEVMKRLVKLGRVSEECGFDTVWLLEHHFTEFGLLGNPYVAAAYLLGATKKLNVGTAAIVLPTAHPVRQLEDVNLLDQMSKGRFRFGICRGLYNKDFRVFGVDMNNTRALMECWYGLIKNGMTEGYMEADNEHIKFHKVKVNPTAYSKGGAPIYVVAESASTTEWAAQFGLPMILSWIINTNEKKAQLELYNEVAREYGHDIHNIDHCLSYITSVDHDSIKAKEICRQFLGHWYDSYVNATTIFDDSDQTKGYGHNKGQWRDFVLKGHKDTNRRIDYSYEINPLGTPKECIDIIQTDIDATGISNICCGFEANGTVDEIIASMKLFQSDVMPFLKETQRSLLY

SEQ ID NO: 42 - protein, 360 aa, Artificial Sequence
  reconstructed sequence
MKFGNFLLTYQPPQFPQTEVMQRLVKLGRVSEECGFDTVWLLEHHFTEFGLLGNPYVAAAYLLGATKKLNVGTAVIVLPTAHPVRQLEDVNLLDQMSKGRFRFGICRGLYNKDFRVFGVDMNNTRALMECWYGLIKRGMTEGYVEADNEHIKFHKVKVNPTAYSQGGAPIYVVAESASTTEWAAQHGLPMILSWIINTNEKKAQLELYNEVAQEHGHDIHNIDHCLSYITSVDHDSIKAKEICRQFLGHWYDSYVNATTIFDDSDQTKGYGFNKGQWRDFVLKGHKDTNRRIDYSYEINPVGTPKECIDIIQTDIDATGISNICCGFEANGTVNEIIASMKLFQSDVMPFLKEKQRSLLY

SEQ ID NO: 43 - protein, 360 aa, Artificial Sequence
  reconstructed sequence
MKFGNFLLTYQPPQFSQTEVMKRLVKLGRVSEECGFDTVWLLEHHFTEFGLLGNPYVAAAYLLGATKKLNVGTAAIVLPTAHPVRQLEDVNLLDQMSKGRFRFGICRGLYNKDFRVFGVDMNNTRALMECWYGLIKNGMTEGYMEADNEHIKFHKVKVNPTAYSQGGAPIYVVAESASTTEWAAQFGLPMILSWIINTNEKKAQLELYNEVAQEYGHDIHNIDHCLSYITSVDHDSIKAKEICRNFLGHWYDSYVNATTIFDDSDQTKGYDFNKGQWRDFVLKGHKDTNRRIDYSYEINPVGTPQECIDIIQTDIDATGISNICCGFEANGTVDEIIASMKLFQSDVMPFLKEKQRSLLY

SEQ ID NO: 44 - protein, 360 aa, Artificial Sequence
  reconstructed sequence
MKFGNFLLTYQPPQFSQTEVMKRLVKLGRVSEECGFDTVWLLEHHFTEFGLLGNPYVAAANLLGATKKLNVGTAAIVLPTAHPVRQLEDVNLLDQMSKGRFRFGICRGLYNKDFRVFGYDMDNTRALMECWYGLIKNGMTEGYMEADNEHIKFPKVHVNPTAYTQGGAPIYVVAESASTTEWAAQFGLPMILSWIVNKNEKIAQLDLYNEVAQEHGHDVHNIDHCLSYITSVDHDSVKAKEVCENFLGHWYDSYVNATTIFDDSDQTKGYGFNKGQWRDFVLKGHKDTNRRIDYSYEINPVGTPKECIDIIQTDIDATGISNICCGFEANGTVDEIIASMKLFQSDVMPFLKEKQRSLLM

SEQ ID NO: 45 - protein, 360 aa, Artificial Sequence
  reconstructed sequence
MKFGNFLLTYQPPQFSQTEVMKRLVKLGRVSEECGFDTVWLLEHHFTEFGLLGNPYVAAANLLGATKKLNVGTAAIVLPTAHPVRQLEDVNLLDQMSKGRFRFGICRGLYNKDFRVFGVDMNNTRALMECWYGLIKNGMTEGYVEADNEHIKFHKVKLNPTAYSRGGAPIYVVAESASTTEWAAQHGLPMILSWIINTNEKKAQLDLYNEVAQEHGHDVHNIDHCLSYITSVDHDSIKAKEICRQFLGHWYDSYVNATTIFDDSDQTKGYGFNKGQWRDFVLKGHKNTNRRIDYSYEINPVGTPQECIDIIQTDIDATGISNICCGFEANGTVDEIIASMKLFQSDVMPFLKETQRSLLF

SEQ ID NO: 46 - protein, 360 aa, Artificial Sequence
  reconstructed sequence
MKFGNFLLTYQPPQFSQTEVMQRLVKLGRVSEECGFDTVWLLEHHFTEFGLLGNPYVAAAHLLGATKKLNVGTAAIVLPTAHPVRQLEDVNLLDQMSKGRFRFGICRGLYNKDFRVFGTDMDNSRALMECWYGLIKNGMTEGYVEADNEHIKFYKVKVGPTAYSQGGAPIYVVAESASTTEWAAQHGLPMILSWIINTNKKIAQLDLYNEVAQEYGHDVHNIDHCLSYITSVDHDSMKAKEICRNFLGHWYDSYVNATTIFDDSDQTKGYDFNKGKWRDFVLKGHKDTNRRIDYSYEINPVETVKEYIDIIQKDIDATGISNICCGFEANGTVDEIIASMKLFQSDVMPFLKEKQRSLLF

SEQ ID NO: 47 - protein, 362 aa, Artificial Sequence
  reconstructed sequence
MRFGNFLLTYQPPQFSQTEVMKRLVKLGRVSEECGFDTVWLLEHHFTEFGLLGNPYVAAAYLLGATKKLNVGTAAIVLPTAHPVRQLEDVNLLDQMSKGRFRFGICRGLYNKDFNVFGVDMNNTRALTECWYGLIKNGMTEGYVEADNEHIKFHKVKVNPTAYTQGGAPIYVVAESASTTEWAAQHGLPMILSWIINTNEKIAQADLYNEVAQEYGHDVHNIDHCLSYITSVDHDSIKAKEICRNFLGHWYDSYVNATTIFDDSDQTKGYDFNKGQWRDFVLKGHKHTNRRIDYSYEINPVGTPQECIDIIQTDIDATGISNICCGFEANGTVDEKIASMKLFQSDVMPFLKETQRSLLMIA

SEQ ID NO: 48 - protein, 360 aa, Artificial Sequence
  reconstructed sequence
MKFGNFLLTYQPPQFSQTEVMKRLVKLGRVSEECGFDTVWLLEHHFTEFGLLGNPYVAAAYLLGATKKLNVGTAAIVLPTAHPVRQLEDVNLLDQMSKGRFRFGICRGLYNKDFRVFGVDMNNTRALMECWYGLIKNGMTEGYVEADNEHIKFHKVKVNPTAYSKGGAPIYVVAESASTTEWAAQHGLPMILSWIINTNEKKAQLELYNEVAQEHGHDVHNIDHCLSYITSVDHDSIKAKEICRNFLGHWYDSYVNATTIFDDSDKTKGYDFNKGQWRDFVLKGHKDTNRRIDYSYEINPVGTPEECIDIIQKDIDATGISNICCGFEANGTVDEIIASMKLFQSDVMPFLKEKQRSLLY

SEQ ID NO: 49 - protein, 360 aa, Artificial Sequence
  reconstructed sequence
MKFGNFLLTYQPPQFSQSEVMQRLVKLGRVSEECGFDTVWLLEHHFTEFGLLGNPYVAAANLLGATKKLNVGTAAIVLPTAHPVRQLEDVNLLDQMSKGRFRFGICRGLYNKDFRVFGTDMDNTRALTECWYGIIKNGMTEGYMEADNEHIKFHKVKVNPTAYSQGGAPIYVVAESASTTEWAAQHGLPMILSWIINNNEKIYQAELYNEVALEYGHDITNIDHCLSYITSVDHDSIKAKEICRDFLGHWYDSYVNATTIFDDSDQTKGYGFNKGQWRDFVLKGHKDTNRRIDYSYEINPVGTPQECIDIIQTDIDATGISNICCGFKANGTVDEIIASMKLFQSDVMPFLKEKQRSLLY

SEQ ID NO: 50 - protein, 360 aa, Artificial Sequence
  reconstructed sequence
MKFGNFLLTYQPPQFSQTEVMQRLVELGRVSEECGFDTVWLLEHHFTEFGLGGNVQVAAAFLLGATKKLNVGTAAIVLPTAHPVRQLEDVNLLDQMSKGRFRFGICRGLYNKDFRVFGVDMNNSRALMEKWYERIKRGITEGYMEADNEHIKFHKVKVNPTAYSQGGAPIYVVATSASTTEWAAQHGLPMILSWIINRNEKIAQIELYNEVAQESGHDIHNIDHCLSYITSVDHDSIKAKEICRNFLGHWYDSYVNATTIFDDSDKTKGYGFNKGQWADFVLKGHKNTNRRIDYSYEINPVGTPKECIDIIQTDIDATGISNICCGFEANGTVDEIIASMKLFQKDVMPFLKETQRSLLF

SEQ ID NO: 51 - protein, 360 aa, Artificial Sequence
  reconstructed sequence
MKFGNFLLTYQPPQFSQGEVMKRLVNLGRVSEECGFDTVWLLEHHFTEFGLLGNPYVAAAYLLGATKKLNVGTAAIVLPTAHPVRQLEDVNLLDQMSKGRFRFGICRGLYNKDFRVFGVDMDNTRALMECWYGLIKEGMTEGYVEADNEHIKFHKVKVNPTAYSKGGAPVYVVAESASTTEWAAQHGLPMILSWIINTNEKKAQLDYYNEVAQEYGHDVHNIDHCLSYITSVDHDSIKAKEICRKFLGHWYDSYVNATTIFDDSDQTKGYDFNKGQWRDFVLKGHKDTNRRIDYSYEINPVGTPEECIDIIQTDIDATGISNICCGFEANGTVDEIIASMKLFQSDVMPFLKEKQRSLLY

SEQ ID NO: 52 - protein, 360 aa, Artificial Sequence
  reconstructed sequence
MKFGNFLLTYQPPQFSQTEVMQRLVKLGRVSEECGFDTVWLLEHHFTEFGLLGNPYVAAAYLLGATKKLNVGTAAIVLPTAHPVRQLEDVNLLDQMSKGRFRFGICRGLYNKDFRVFGTDMDNSRALMECWYGLIKNGMTEGYVEADNEHIKFHKVKVNPTAYSQGGAPVYVVAESASTTEWAAQHGLPMILSWIINTNEKKAQLELYNEVAQEYGHDIHNIDHCLSYITSVDHDSIKAKEICRNFLGHWYDSYVNATTIFDDSDQTKGYDFNKGQWRDFVLKGHKDTNRRIDYSYEINPVGTPQECIDIIQTDIDATGISNICCGFEANGTVDEIIASMKLFQSDVMPFLKEKQRSLLY

SEQ ID NO: 53 - DNA, 1172 bp, Artificial Sequence
  reconstructed sequence
caattttcgtactgaaacatcttaatcatgcacaggagactttctaatgaaatttggaaactttttgcttacataccaacctccccaattttctcaaacagaggtaatgaaacgtttggttaaattaggtcgcgtgtctgaggagtgtggttttgataccgtatggttactggagcatcatttcacggagtttggtttgcttggtaacccttatgtcgctgctgcatatttacttggcgcgactaaaaaattgaatgtaggaactgccgctattgttcttcccacagcccatccagtacgccaacttgaagatgtgaatttattggatcaaatgtcaaaaggacgatttcggtttggtatttgccgagggctttacaacaaggactttcgcgtattcggcgttgatatgaataacacacgcgccttaatggaatgctggtacgggctgataaagaatggcatgacagagggatatgtggaagctgataatgaacatatcaagttccataaggtaaaagtaaaccccaccgcgtatagccagggtggcgcaccggtttatgtggtggctgaatcagcttcgacgactgagtgggctgctcaacatggcctaccgatgatattaagttggattataaatactaacgaaaagaaagcacaacttgagctttataatgaagtggctcaagaatatgggcacgatgttcataatatcgaccattgcttatcatatataacatctgtagatcatgactcaattaaagcgaaagagatttgccggaactttctggggcattggtatgattcttatgtgaatgctacgactatttttgatgattcagaccaaacaaaaggttatgatttcaataaagggcagtggcgtgactttgtattaaaaggacataaagatactaatcgccgtattgattacagttacgaaatcaatcccgtgggaacgccgaaggaatgtattgacataattcaaaccgacattgatgctacaggaatatcaaatatttgttgtggatttgaagctaatggaacagtagacgaaattattgcttccatgaagctcttccagtctgatgtcatgccatttcttaaagaaaaacaacgttcgctattatattgaggatcggttgtcgagtaaggatctccaggcatcaaataaaacg

SEQ ID NO: 54 - DNA, 1169 bp, Artificial Sequence
  reconstructed sequence
caattttcgtactgaaacatcttaatcatgcacaggagactttctaatgaaatttggaaactttttgcttacataccaacctccccaattttctcaaacagaggtaatgcaacgtttggttaacttaggtcgcgcctctgaggagtgtggttttgataccgtatggttactggagcatcatttcacggagtttggtttgcttggtaacccttatgtcgctgctgcatatttacttggcgcgactaaacacttgaatgtaggaactgccgctattgttcttcccacagcccatccagtacgccaacttgaagatgtgaatttattggatcaaatgtcaaaaggacgatttcggtttggtatttgccgagggctttacaacaaggactttaatgtattcggcgttgatatgaataacacacgcgccttaactgaatgctggtacgggctgataaagaatggcatgacagagggatatatggaagctgataatgaacatatcaagttccataaggtaaaagtaaaccccaccgcgtatagcaagggtggcgcaccggtttatgtggtggctgaatcagcttcgacgactgagtgggctgctcaacatggcctaccgatgatattaagttggattataaatactaacgaaaagaaagcacaaattgatctttataatgaagtggctcaagaacacgggcacgatgttcataatatcgaccattgcttatcatatataacatctgtagatcatgactcaaagaaagcgaaagagatttgccgggattttctggggcattggtatgattcttatgtgaatgctacgactatttttgatgattcagaccaaacaaaaggttatggcttcaataaagggcagtggcatgactttgtattaaaaggacataaagatactaatcgccgtgttgattacagttacgaaatcaatcccgtgggaacgccgcaggaatgtattgacataattcaaaccgacattgatgctacaggaatatcaaatatttgttgtggatttgaagctaatggaacagtagacgaaattattgcttccatgaagctcttccagtctgatgtcatgccatttcttaaagaaaaacaacgttcgctattatgaggatcggttgtcgagtaaggatctccaggcatcaaataaaacg

SEQ ID NO: 55 - DNA, 1169 bp, Artificial Sequence
  reconstructed sequence
caattttcgtactgaaacatcttaatcatgcacaggagactttctaatgaaatttggaaactttttgcttacataccaacctccccaattttctcaaacagaggtaatgcaacgtttggttaaattaggtcgcgtgtctgaggagtgtggttttgataccgtatggttactggagcatcatttcacggagtttggtttgcttggtaacccttatgtcgctgctgcatatttacttggcgcgactaaaaaattgaatgtaggaactgccgctattgttcttcccacagcccatccagtacgccaacttgaagatgtgaatttattggatcaaatgtcaaaaggacgatttcggtttggtatttgccgagggctttacaacaaggactttcgcgtattcggcgttgatatgaataacacacgcgccttaatggaatgctggtacgggctgataaagaatggcatgacagagggatatatggaagctgataatgaacatatcaagttccataaggtaaaagtaaaccccaccgcgtatacacagggtggcgcaccgatttatgtggtggctgaatcagcttcgacgactgagtgggctgctcaatttggcctaccgatgatattaagttggattataaatactaacgaaaagatcgcacaacttgagctttataatgaagtggctcaagaatatgggcacgatgttcataatatcgaccattgcttatcatatataacatctgtagatcatgactcaattaaagcgaaagagatttgccggcaatttctggggcattggtatgattcttatgtgaatgctacgactatttttgatgattcagaccaaacaaaaggttatgatttcaataaagggcagtggcgtgactttgtattaaaaggacataaagatactaatcgccgtattgattacagttacgaaatcaatcccgtgggaacgccgaaggaatgtattgacataattcaaaccgacattgatgctacaggaatatcaaatatttgttgtggatttgaagctaatggaacagtagacgaaattattgcttccatgaagctcttccagtctgatgtcatgccatttcttaaagaaaaacaacgttcgctattatgaggatcggttgtcgagtaaggatctccaggcatcaaataaaacg

SEQ ID NO: 56 - DNA, 1169 bp, Artificial Sequence
  reconstructed sequence
caattttcgtactgaaacatcttaatcatgcacaggagactttctaatgaaatttggaaactttttgcttacataccaacctccccaattttctcaaacagaggtaatgcaacgtttggttaaattaggtcgcgtgtctgaggagtgtggttttgataccgtatggttactggagcatcatttcacggagtttggtttgcttggtaacccttatgtcgctgctgcatatttacttggcgcgactaaaaaattgaatgtaggaactgccgctattgttcttcccacagcccatccagtacgccaacttgaagatgtgaatttattggatcaaatgtcaaaaggacgatttcggtttggtatttgccgagggctttacaacaaggactttcgcgtattcggcgttgatatgaataacacacgcgccttaatggaatgctggtacgggctgataaagaatggcatgacagagggatatgtggaagctgataatgaacatatcaagttccataaggtaaaagtaaaccccaccgcgtatagccagggtggcgcaccggtttatgtggtggctgaatcagcttcgacgactgagtgggctgctcaacatggcctaccgatgatattaagttggattataaatactaacgaaaagatcgcacaaattgagctttataatgaagtggctcaagaatatgggcacgatattcataatatcgaccattgcttatcatatataacatctgtagatcatgactcaattaaagcgaaagagatttgccggaactttctggggcattggtatgattcttatgtgaatgctacgactatttttgatgattcagacaagacaaaaggttatggcttcaataaagggcagtggcgtgactttgtattaaaaggacataaagatactaatcgccgtattgattacagttacgaaatcaatcccgtgggaacgccgaaggaatgtattgacataattcaaaccgacattgatgctacaggaatatcaaatatttgttgtggatttgaagctaatggaacagtagacgaaattattgcttccatgaagctcttccagtctgatgtcatgccatttcttaaagaaacgcaacgttcgctattatgaggatcggttgtcgagtaaggatctccaggcatcaaataaaacg

SEQ ID NO: 57 - DNA, 1172 bp, Artificial Sequence
  reconstructed sequence
caattttcgtactgaaacatcttaatcatgcacaggagactttctaatgaaatttggaaactttttgcttacataccaacctccccaactggaccaatccgaggtaatggcgcgtttggttaaattaggtcgcgtgtctgaggagtgtggttttgataccgtatggttactggagcatcatttcacggagtttggtttgcttggtaacccttatgtcgctgctgcatatttacttggcgcgactaaaaaattgaatgtaggaactgccgctattgttcttcccacagcccatccagtacgccaacttgaagatgtgaatttattggatcaaatgtcaaaaggacgatttcggtttggtatttgccgagggctttacaacaaggactttcgcgtattcggcgttgatatgaataacagtcgcgccttaatggaatgctggtacgacctgataaaggaaggcatgacagagggatatgtggaagctgatacggaacatatcaagttccataaggtaaaacatttgcccaccgcgtatagccagggtggcgcaccggtttatgtggtggctgaatcagcttcgacgactgagtgggctgctcaacatggcctaccgatgatattaagttggattataaatactaacgaaaagaaagcacaacttgagctttataatgaagtggctcaagaatatgggcacgatattcataatatcgaccattgcttatcatatataacatctgtagatcatgactcaattcgtgcgaaagagaaatgcgtcaaccatctggggcattggtatgattcttatgtgaatgctacgactatttttgatgattcagaccaaacaaaaggttatggcttcaataaagggcagtggcgtgactttgtattaaaaggacataaagatactaatcgccgtattgattacagttacgaaatcaatcccgtgggaacgccgaacgaatgtattgacataattcaaaccgacattgatgctacaggaatatcaaatatttgttgtggatttgaagctaatggaacagtagacgaacgtattgcttccatgttgctcttccagtctgatgtcatgccatttcttaaagaaaaacaacgttcgctattatattgaggatcggttgtcgagtaaggatctccaggcatcaaataaaacg

SEQ ID NO: 58 - DNA, 1172 bp, Artificial Sequence
  reconstructed sequence
caattttcgtactgaaacatcttaatcatgcacaggagactttctaatgaaatttggaaactttttgcttacataccaacctccccaattttctcaaacagaggtaatgcaacgtttggttaaattaggtcgcgtgtctgaggagtgtggttttgataccgtatggttactggagcatcatttcacggagtttggtttgcttggtaacccttatgtcgctgctgcatatttacttggcgcgactaaaaaattgaatgtaggaactgccgctattgttcttcccacagcccatccagtacgccaacttgaagatgtgaatttattggatcaaatgtcaaaaggacgatttcggtttggtatttgccgagggctttacaacaaggactttcgcgtattcggcgttgatatgaataacacacgcgccttaatggaatgctggtacgggctgataaagaatggcatgacagagggatatgtggaagctgataatgaacatatcaagttccataaggtaaaagtaaaccccaccgcgtatagccagggtggcgcaccggtttatgtggtggctgaatcagcttcgacgactgagtgggctgctcaatttggcctaccgatgatattaagttggattataaatactaacgaaaagaaagcacaacttgagctttataatgaagtggctcaagaatatgggcacgatattcataatatcgaccattgcttatcatatataacatctgtagatcatgactcaattaaagcgaaagagatttgccggaactttctggggcattggtatgattcttatgtgaatgctacgactatttttgatgattcagaccaaacaaaaggttatggcttcaataaagggcagtggcgtgactttgtattaaaaggacataaaaatactaatcgccgtattgattacagttacgaaatcaatcccgtgggaacgccgaaggaatgtattgacataattcaaaccgacattgatgctacaggaatatcaaatatttgttgtggatttgaagctaatggaacagtagacgaaattattgcttccatgaagctcttccagtctgatgtcatgccatttcttaaagaaaaacaacgttcgctattatattgaggatcggttgtcgagtaaggatctccaggcatcaaataaaacg

SEQ ID NO: 59 - DNA, 1169 bp, Artificial Sequence
  reconstructed sequence
caattttcgtactgaaacatcttaatcatgcacaggagactttctaatgaaatttggaaactttttgcttacataccaacctccccaattttctcaaacagaggtaatgaaacgtttggttaaattaggtcgcgtgtctgaggagtgtggttttgataccgtatggttactggagcatcatttcacggagtttggtttgcttggtaacccttatgtcgctgctgcatatttacttggcgcgactaaaaaattgaatgtaggaactgccgctattgttcttcccacagcccatccagtacgccaacttgaagatgtgaatttattggatcaaatgtcaaaaggacgatttcggtttggtatttgccgagggctttacaacaaggactttcgcgtattcggcgttgatatggataacacacgcgccttaatggaatgctggtacgggctgataaagaatggcatgacagagggatatgtggaagctgataatgaacatatcaagttccataaggtaaaagtaaaccccaccgcgtatagccagggtggcgcaccgatttatgtggtggctgaatcagcttcgacgactgagtgggctgctcaacatggcctaccgatgatattaagttggattataaatactaacgaaaagaaagcacaacttgagctttataatgaagtggctcaagaacacgggcacgatgttcataatatcgaccattgcttatcatatataacatctgtagatcatgactcaattaaagcgaaagagatttgccggaactttctggggcattggtatgattcttatgtgaatgctacgactatttttgatgattcagaccaaacaaaaggttatggcttcaataaagggcagtggcgtgactttgtattaaaaggacataaagatactaatcgccgtattgattacagttacgaaatcaatcccgtgggaacgccgaaggaatgtattgacataattcaaaccgacattgatgctacaggaatatcaaatatttgttgtggatttgaagctaatggaacagtagacgaaattattgcttccatgaagctcttccagtctgatgtcatgccatttcttaaagaaaaacaacgttcgctattatgaggatcggttgtcgagtaaggatctccaggcatcaaataaaacg

SEQ ID NO: 60 - DNA, 1172 bp, Artificial Sequence
  reconstructed sequence
caattttcgtactgaaacatcttaatcatgcacaggagactttctaatgaaatttggaaactttttgcttacataccaacctccccaattttctcaaacagaggtaatgcaacgtttggttaaattaggtcgcgtgtctgaggagtgtggttttgataccgtatggttactggagcatcatttcacggagtttggtttgcttggtaacccttatgtcgctgctgcatatttacttggcgcgactaaaaaattgaatgtaggaactgccgctattgttcttcccacagcccatccagtacgccaacttgaagatgtgaatttattggatcaaatgtcaaaaggacgatttcggtttggtatttgccgagggctttacaacaaggactttcgcgtattcggcgttgatatgaataacacacgcgccttaatggaatgctggtacgggctgataaagaatggcatgacagagggatatatggaagctgataatgaacatatcaagttccataaggtaaaagtaaaccccaccgcgtatagccagggtggcgcaccggtttatgtggtggctgaatcagcttcgacgactgagtgggctgctcaacatggcctaccgatgatattaagttggattataaatactaacgaaaagaaagcacaacttgagctttataatgaagtggctcaagaacacgggcacgatattcataatatcgaccattgcttatcatatataacatctgtagatcatgactcaattaaagcgaaagagatttgccggaactttctggggcattggtatgattcttatgtgaatgctacgactatttttgatgattcagaccaaacaaaaggttatgatttcaataaagggcagtggcgtgactttgtattaaaaggacataaagatactaatcgccgtattgattacagttacgaaatcaatcccgtgggaacgccgaaggaatgtattgacataattcaaaccgacattgatgctacaggaatatcaaatatttgttgtggatttgaagctaatggaacagtagacgaaattattgcttccatgaagctcttccagtctgatgtcatgccatttcttaaagaaaaacaacgttcgctattatattgaggatcggttgtcgagtaaggatctccaggcatcaaataaaacg

SEQ ID NO: 61 - DNA, 1172 bp, Artificial Sequence
  reconstructed sequence
caattttcgtactgaaacatcttaatcatgcacaggagactttctaatgaaatttggaaactttttgcttacataccaacctccccaactgccgcaaacagaggtaatgaaacgtttggttaaattaggtcgcgtgtctgagggttgtggttttgataccgtatggttactggagcatcatttcacggagtttggtttgcttggtaacccttatgtcgctgctgcacatttacttggcgcgactaaaaaattgaatgtaggaactgccgctattgttcttcccacagcccatccaattcgccaacttgaagatgtgaatttattggatcaaatgtcaaaaggacgatttcggtttggtatttgccgagggctttacaacaaggactttcgcgtattcggcacagatatgaataacagtcgcgtgttaatggaatgctggtacgggctgataaagaatggcatgacagagggatatatggaagctgataatgaacatatcaagttccataaggtaaaagtaaaccccaccgcgtatagcagaggtggcgcaccggtttatgtggtggctgaatcagcttcgacgactgagtgggctgctcaatttggcctaccgatgatattaagttggattataaatactaacgaaaagaaagcacaagctgagctttataatgaagtggctctcgaatatgggcgtgatattcataatatcgaccattgcttatcatatataacatctgtagatcatgactcaattaaagcgaaagagatttgccggaactttctggggcattggtatgattcttatgtgaatgctacgactatttttgatgattcagaccaaacaaaaggttatgatttcaataaagggcagtggcgtgactttgtattaaaaggacataaagatactaatcgccgtattgattacagttacgaaatcaatcccgtgggaacgccggaagaatgtattgacataattcaaaccgacattgatgctacaggaatatcaaatatttgttgtggatttgaagctaatggaacagtagacgaaattattgcttccatgaagctcttccagtctgatgtcatgccatttcttaaagaaaaacaacgttcgctattatattgaggatcggttgtcgagtaaggatctccaggcatcaaataaaacg

SEQ ID NO: 62 - DNA, 1172 bp, Artificial Sequence
  reconstructed sequence
caattttcgtactgaaacatcttaatcatgcacaggagactttctaatgaaatttggaaactttttgcttacataccaacctccccaattttctcaaacagaggtaatgaaacgtttggttaaattaggtcgcgtgtctgaggagtgtggttttgataccgtatggttactggagcatcatttcacggagtttggtttgcttggtaacccttatgtcgctgctgcatatttacttggcgcgactaaaaaattgaatgtaggaactgccgctattgttcttcccacagcccatccagtacgccaacttgaagatgtgaatttattggatcaaatgtcaaaaggacgatttcggtttggtatttgccgagggctttacaacaaggactttcgcgtattcggcgttgatatgaataacagtcgcgccttaatggaatgctggtacgggctgataaagaatggcatgacagagggatatgtggaagctgataatgaacatatcaagttccataaggtaaaagtaaaccccaccgcgtatagccagggtggcgcaccgatttatgtggtggctgaatcagcttcgacgactgagtgggctgctcaacatggcctaccgatgatattaagttggattataaatactaacgaaaagaaagcacaacttgagttttataatgaagtggctcaagaatatgggcacgatattcataatatcgaccattgcttatcatatataacatctgtagatcatgactcaattaaagcgaaagagatttgccggaactttctggggcattggtatgattcttatgtgaatgctacgactatttttgatgattcagaccaaacaaaaggttatggcttcaataaagggcagtggcgtgactttgtattaaaaggacataaaaatactaatcgccgtattgattacagttacgaaatcaatcccgtgggaacgccgaaggaatgtattgacataattcaaaccgacattgatgctacaggaatatcaaatatttgttgtggatttgaagctaatggaacagtagacgaaattattgcttccatgaagctcttccagtctgatgtcatgccatttcttaaagaaaaacaacgttcgctattatattgaggatcggttgtcgagtaaggatctccaggcatcaaataaaacg

SEQ ID NO: 63 - DNA, 1172 bp, Artificial Sequence
  reconstructed sequence
caattttcgtactgaaacatcttaatcatgcacaggagactttctaatgaaatttggaaactttttgcttacataccaacctcccgaattttctcaaacagaggtaatgaaacgtttggttaaattaggtcgcgtgtctgaggagtgtggttttgatgaagtatggttactggagcatcatttcacggagtttggtttgcttggtaacccttatgtcgctgctgcacatttacttggcgcgactaaaaaattgaatgtaggaactgccgctattgttcttcccacagcccatccagtacgccaacttgaagatgtgaatttattggatcaaatgtcaaaaggacgatttcggtttggtatttgccgagggctttacaacaaggactttcgcgtattcggcgttgatatgaataacagtcgcgtgttaatggaatgctggtacgggctgatgaagaatggcatgacagagggatatatggaagctgataatgaacatatcaagttccataaggtaaaagtaaaccccaccgcgtatacacagggtggcgcaccgatttatgtggtggctgaatcagcttcgacgactgagtgggctgctcaacatggcctaccgatgatattaagttggattataaataataacgaaaagatctatcaagctaaattttataatgaagtggctcaagaatccgggcacgatattcataatatcgaccattgcttatcatatataacatctgtagatcatgactcaattaaagcgaaagagatttgccggaactttctggggcattggtatgattcttatgtgaatgctacgactatttttgatgattcagacaagacaaaaggttatgatttcaataaagggcagtggcgtgactttgtattaaaaggacataaagatactaatcgccgtattgattacagttacgaaatcaatcccgtgggaacgccgaaggaatgtattgacataattcaaaccgacattgatgctacaggaatatcaataaactgttgtggatttgaagctaatggaacagtagacgaaattattgcttccatgaagctcttccagtctgatgtcatgccatttcttaaagaaaaacaacgttcgctattatattgaggatcggttgtcgagtaaggatctccaggcatcaaataaaacg

SEQ ID NO: 64 - DNA, 1172 bp, Artificial Sequence
  reconstructed sequence
caattttcgtactgaaacatcttaatcatgcacaggagactttctaatgaaatttggaaactttttgcttacataccaacctccccaattttctcaaacagaggtaatgaaacgtttggttaaattaggtcgcgtgtctgaggagtgtggttttgataccgtatggttactggagcatcatttcacggagtttggtttgcttggtaacccttatgtcgctgctgcatatttacttggcgcgactaaaaaattgaatgtaggaactgccgctattgttcttcccacagcccatccagtacgccaacttgaagatgtgaatttattggatcaaatgtcaaaaggacgatttcggtttggtatttgccgagggctttacaacaaggactttcgcgtattcggcgttgatatgaataacacacgcgccttaatggaatgctggtacgggctgataaagaatggcatgacagagggatatatggaagctgataatgaacatatcaagttccataaggtaaaagtaaaccccaccgcgtatagcaagggtggcgcaccgatttatgtggtggctgaatcagcttcgacgactgagtgggctgctcaatttggcctaccgatgatattaagttggattataaatactaacgaaaagaaagcacaacttgagctttataatgaagtggctcgtgaatatgggcacgatattcataatatcgaccattgcttatcatatataacatctgtagatcatgactcaattaaagcgaaagagatttgccggcaatttctggggcattggtatgattcttatgtgaatgctacgactatttttgatgattcagaccaaacaaaaggttatggccacaataaagggcagtggcgtgactttgtattaaaaggacataaagatactaatcgccgtattgattacagttacgaaatcaatccccttggaacgccgaaggaatgtattgacataattcaaaccgacattgatgctacaggaatatcaaatatttgttgtggatttgaagctaatggaacagtagacgaaattattgcttccatgaagctcttccagtctgatgtcatgccatttcttaaagaaacgcaacgttcgctattatattgaggatcggttgtcgagtaaggatctccaggcatcaaataaaacg

SEQ ID NO: 65 - DNA, 1172 bp, Artificial Sequence
  reconstructed sequence
caattttcgtactgaaacatcttaatcatgcacaggagactttctaatgaaatttggaaactttttgcttacataccaacctccccaatttccgcaaacagaggtaatgcaacgtttggttaaattaggtcgcgtgtctgaggagtgtggttttgataccgtatggttactggagcatcatttcacggagtttggtttgcttggtaacccttatgtcgctgctgcatatttacttggcgcgactaaaaaattgaatgtaggaactgccgtcattgttcttcccacagcccatccagtacgccaacttgaagatgtgaatttattggatcaaatgtcaaaaggacgatttcggtttggtatttgccgagggctttacaacaaggactttcgcgtattcggcgttgatatgaataacacacgcgccttaatggaatgctggtacgggctgataaagcgtggcatgacagagggatatgtggaagctgataatgaacatatcaagttccataaggtaaaagtaaaccccaccgcgtatagccagggtggcgcaccgatttatgtggtggctgaatcagcttcgacgactgagtgggctgctcaacatggcctaccgatgatattaagttggattataaatactaacgaaaagaaagcacaacttgagctttataatgaagtggctcaagaacacgggcacgatattcataatatcgaccattgcttatcatatataacatctgtagatcatgactcaattaaagcgaaagagatttgccggcaatttctggggcattggtatgattcttatgtgaatgctacgactatttttgatgattcagaccaaacaaaaggttatggcttcaataaagggcagtggcgtgactttgtattaaaaggacataaagatactaatcgccgtattgattacagttacgaaatcaatcccgtgggaacgccgaaggaatgtattgacataattcaaaccgacattgatgctacaggaatatcaaatatttgttgtggatttgaagctaatggaacagtaaatgaaattattgcttccatgaagctcttccagtctgatgtcatgccatttcttaaagaaaaacaacgttcgctattatattgaggatcggttgtcgagtaaggatctccaggcatcaaataaaacg

SEQ ID NO: 66 - DNA, 1172 bp, Artificial Sequence
  reconstructed sequence
caattttcgtactgaaacatcttaatcatgcacaggagactttctaatgaaatttggaaactttttgcttacataccaacctccccaattttctcaaacagaggtaatgaaacgtttggttaaattaggtcgcgtgtctgaggagtgtggttttgataccgtatggttactggagcatcatttcacggagtttggtttgcttggtaacccttatgtcgctgctgcatatttacttggcgcgactaaaaaattgaatgtaggaactgccgctattgttcttcccacagcccatccagtacgccaacttgaagatgtgaatttattggatcaaatgtcaaaaggacgatttcggtttggtatttgccgagggctttacaacaaggactttcgcgtattcggcgttgatatgaataacacacgcgccttaatggaatgctggtacgggctgataaagaatggcatgacagagggatatatggaagctgataatgaacatatcaagttccataaggtaaaagtaaaccccaccgcgtatagccagggtggcgcaccgatttatgtggtggctgaatcagcttcgacgactgagtgggctgctcaatttggcctaccgatgatattaagttggattataaatactaacgaaaagaaagcacaacttgagctttataatgaagtggctcaagaatatgggcacgatattcataatatcgaccattgcttatcatatataacatctgtagatcatgactcaattaaagcgaaagagatttgccggaactttctggggcattggtatgattcttatgtgaatgctacgactatttttgatgattcagaccaaacaaaaggttatgatttcaataaagggcagtggcgtgactttgtattaaaaggacataaagatactaatcgccgtattgattacagttacgaaatcaatcccgtgggaacgccgcaggaatgtattgacataattcaaaccgacattgatgctacaggaatatcaaatatttgttgtggatttgaagctaatggaacagtagacgaaattattgcttccatgaagctcttccagtctgatgtcatgccatttcttaaagaaaaacaacgttcgctattatattgaggatcggttgtcgagtaaggatctccaggcatcaaataaaacg

SEQ ID NO: 67 - DNA, 1172 bp, Artificial Sequence
  reconstructed sequence
caattttcgtactgaaacatcttaatcatgcacaggagactttctaatgaaatttggaaactttttgcttacataccaacctccccaattttctcaaacagaggtaatgaaacgtttggttaaattaggtcgcgtgtctgaggagtgtggttttgataccgtatggttactggagcatcatttcacggagtttggtttgcttggtaacccttatgtcgctgctgcaaatttacttggcgcgactaaaaaattgaatgtaggaactgccgctattgttcttcccacagcccatccagtacgccaacttgaagatgtgaatttattggatcaaatgtcaaaaggacgatttcggtttggtatttgccgagggctttacaacaaggactttcgcgtattcggctatgatatggataacacacgcgccttaatggaatgctggtacgggctgataaagaatggcatgacagagggatatatggaagctgataatgaacatatcaagttccccaaggtacatgtaaaccccaccgcgtatacacagggtggcgcaccgatttatgtggtggctgaatcagcttcgacgactgagtgggctgctcaatttggcctaccgatgatattaagttggattgtgaataaaaacgaaaagatcgcacaacttgatctttataatgaagtggctcaagaacacgggcacgatgttcataatatcgaccattgcttatcatatataacatctgtagatcatgactcagttaaagcgaaagaggtctgcgaaaactttctggggcattggtatgattcttatgtgaatgctacgactatttttgatgattcagaccaaacaaaaggttatggcttcaataaagggcagtggcgtgactttgtattaaaaggacataaagatactaatcgccgtattgattacagttacgaaatcaatcccgtgggaacgccgaaggaatgtattgacataattcaaaccgacattgatgctacaggaatatcaaatatttgttgtggatttgaagctaatggaacagtagacgaaattattgcttccatgaagctcttccagtctgatgtcatgccatttcttaaagaaaaacaacgttcgctattaatgtgaggatcggttgtcgagtaaggatctccaggcatcaaataaaacg

SEQ ID NO: 68 - DNA, 1172 bp, Artificial Sequence
  reconstructed sequence
caattttcgtactgaaacatcttaatcatgcacaggagactttctaatgaaatttggaaactttttgcttacataccaacctccccaattttctcaaacagaggtaatgaaacgtttggttaaattaggtcgcgtgtctgaggagtgtggttttgataccgtatggttactggagcatcatttcacggagtttggtttgcttggtaacccttatgtcgctgctgcaaatttacttggcgcgactaaaaaattgaatgtaggaactgccgctattgttcttcccacagcccatccagtacgccaacttgaagatgtgaatttattggatcaaatgtcaaaaggacgatttcggtttggtatttgccgagggctttacaacaaggactttcgcgtattcggcgttgatatgaataacacacgcgccttaatggaatgctggtacgggctgataaagaatggcatgacagagggatatgtggaagctgataatgaacatatcaagttccataaggtaaaactgaaccccaccgcgtatagcagaggtggcgcaccgatttatgtggtggctgaatcagcttcgacgactgagtgggctgctcaacatggcctaccgatgatattaagttggattataaatactaacgaaaagaaagcacaacttgatctttataatgaagtggctcaagaacacgggcacgatgttcataatatcgaccattgcttatcatatataacatctgtagatcatgactcaattaaagcgaaagagatttgccggcaatttctggggcattggtatgattcttatgtgaatgctacgactatttttgatgattcagaccaaacaaaaggttatggcttcaataaagggcagtggcgtgactttgtattaaaaggacataaaaatactaatcgccgtattgattacagttacgaaatcaatcccgtgggaacgccgcaggaatgtattgacataattcaaaccgacattgatgctacaggaatatcaaatatttgttgtggatttgaagctaatggaacagtagacgaaattattgcttccatgaagctcttccagtctgatgtcatgccatttcttaaagaaacgcaacgttcgctattattctgaggatcggttgtcgagtaaggatctccaggcatcaaataaaacg

SEQ ID NO: 69 - DNA, 1172 bp, Artificial Sequence
  reconstructed sequence
caattttcgtactgaaacatcttaatcatgcacaggagactttctaatgaaatttggaaactttttgcttacataccaacctccccaattttctcaaacagaggtaatgcaacgtttggttaaattaggtcgcgtgtctgaggagtgtggttttgataccgtatggttactggagcatcatttcacggagtttggtttgcttggtaacccttatgtcgctgctgcacatttacttggcgcgactaaaaaattgaatgtaggaactgccgctattgttcttcccacagcccatccagtacgccaacttgaagatgtgaatttattggatcaaatgtcaaaaggacgatttcggtttggtatttgccgagggctttacaacaaggactttcgcgtattcggcacagatatggataacagtcgcgccttaatggaatgctggtacgggctgataaagaatggcatgacagagggatatgtggaagctgataatgaacatatcaagttctataaggtaaaagtagggcccaccgcgtatagccagggtggcgcaccgatttatgtggtggctgaatcagcttcgacgactgagtgggctgctcaacatggcctaccgatgatattaagttggattataaatactaacaaaaagatcgcacaacttgatctttataatgaagtggctcaagaatatgggcacgatgttcataatatcgaccattgcttatcatatataacatctgtagatcatgactcaatgaaagcgaaagagatttgccggaactttctggggcattggtatgattcttatgtgaatgctacgactatttttgatgattcagaccaaacaaaaggttatgatttcaataaagggaagtggcgtgactttgtattaaaaggacataaagatactaatcgccgtattgattacagttacgaaatcaatcccgtggaaacggtaaaggaatacattgacataattcaaaaagacattgatgctacaggaatatcaaatatttgttgtggatttgaagctaatggaacagtagacgaaattattgcttccatgaagctcttccagtctgatgtcatgccatttcttaaagaaaaacaacgttcgctattattctgaggatcggttgtcgagtaaggatctccaggcatcaaataaaacg

SEQ ID NO: 70 - DNA, 1178 bp, Artificial Sequence
  reconstructed sequence
caattttcgtactgaaacatcttaatcatgcacaggagactttctaatgcgctttggaaactttttgcttacataccaacctccccaattttctcaaacagaggtaatgaaacgtttggttaaattaggtcgcgtgtctgaggagtgtggttttgataccgtatggttactggagcatcatttcacggagtttggtttgcttggtaacccttatgtcgctgctgcatatttacttggcgcgactaaaaaattgaatgtaggaactgccgctattgttcttcccacagcccatccagtacgccaacttgaagatgtgaatttattggatcaaatgtcaaaaggacgatttcggtttggtatttgccgagggctttacaacaaggactttaatgtattcggcgttgatatgaataacacacgcgccttaactgaatgctggtacgggctgataaagaatggcatgacagagggatatgtggaagctgataatgaacatatcaagttccataaggtaaaagtaaaccccaccgcgtatacacagggtggcgcaccgatttatgtggtggctgaatcagcttcgacgactgagtgggctgctcaacatggcctaccgatgatattaagttggattataaatactaacgaaaagatcgcacaagctgatctttataatgaagtggctcaagaatatgggcacgatgttcataatatcgaccattgcttatcatatataacatctgtagatcatgactcaattaaagcgaaagagatttgccggaactttctggggcattggtatgattcttatgtgaatgctacgactatttttgatgattcagaccaaacaaaaggttatgatttcaataaagggcagtggcgtgactttgtattaaaaggacataaacacactaatcgccgtattgattacagttacgaaatcaatcccgtgggaacgccgcaggaatgtattgacataattcaaaccgacattgatgctacaggaatatcaaatatttgttgtggatttgaagctaatggaacagtagacgaaaaaattgcttccatgaagctcttccagtctgatgtcatgccatttcttaaagaaacgcaacgttcgctattaatgatcgcgtgaggatcggttgtcgagtaaggatctccaggcatcaaataaaacg

SEQ ID NO: 71 - DNA, 1172 bp, Artificial Sequence
  reconstructed sequence
caattttcgtactgaaacatcttaatcatgcacaggagactttctaatgaaatttggaaactttttgcttacataccaacctccccaattttctcaaacagaggtaatgaaacgtttggttaaattaggtcgcgtgtctgaggagtgtggttttgataccgtatggttactggagcatcatttcacggagtttggtttgcttggtaacccttatgtcgctgctgcatatttacttggcgcgactaaaaaattgaatgtaggaactgccgctattgttcttcccacagcccatccagtacgccaacttgaagatgtgaatttattggatcaaatgtcaaaaggacgatttcggtttggtatttgccgagggctttacaacaaggactttcgcgtattcggcgttgatatgaataacacacgcgccttaatggaatgctggtacgggctgataaagaatggcatgacagagggatatgtggaagctgataatgaacatatcaagttccataaggtaaaagtaaaccccaccgcgtatagcaagggtggcgcaccgatttatgtggtggctgaatcagcttcgacgactgagtgggctgctcaacatggcctaccgatgatattaagttggattataaatactaacgaaaagaaagcacaacttgagctttataatgaagtggctcaagaacacgggcacgatgttcataatatcgaccattgcttatcatatataacatctgtagatcatgactcaattaaagcgaaagagatttgccggaactttctggggcattggtatgattcttatgtgaatgctacgactatttttgatgattcagacaagacaaaaggttatgatttcaataaagggcagtggcgtgactttgtattaaaaggacataaagatactaatcgccgtattgattacagttacgaaatcaatcccgtgggaacgccggaagaatgtattgacataattcaaaaagacattgatgctacaggaatatcaaatatttgttgtggatttgaagctaatggaacagtagacgaaattattgcttccatgaagctcttccagtctgatgtcatgccatttcttaaagaaaaacaacgttcgctattatattgaggatcggttgtcgagtaaggatctccaggcatcaaataaaacg

SEQ ID NO: 72 - DNA, 1172 bp, Artificial Sequence
  reconstructed sequence
caattttcgtactgaaacatcttaatcatgcacaggagactttctaatgaaatttggaaactttttgcttacataccaacctccccaattttctcaatccgaggtaatgcaacgtttggttaaattaggtcgcgtgtctgaggagtgtggttttgataccgtatggttactggagcatcatttcacggagtttggtttgcttggtaacccttatgtcgctgctgcaaatttacttggcgcgactaaaaaattgaatgtaggaactgccgctattgttcttcccacagcccatccagtacgccaacttgaagatgtgaatttattggatcaaatgtcaaaaggacgatttcggtttggtatttgccgagggctttacaacaaggactttcgcgtattcggcacagatatggataacacacgcgccttaactgaatgctggtacgggattataaagaatggcatgacagagggatatatggaagctgataatgaacatatcaagttccataaggtaaaagtaaaccccaccgcgtatagccagggtggcgcaccgatttatgtggtggctgaatcagcttcgacgactgagtgggctgctcaacatggcctaccgatgatattaagttggattataaataataacgaaaagatctatcaagctgagctttataatgaagtggctctcgaatatgggcacgatattacgaatatcgaccattgcttatcatatataacatctgtagatcatgactcaattaaagcgaaagagatttgccgggattttctggggcattggtatgattcttatgtgaatgctacgactatttttgatgattcagaccaaacaaaaggttatggcttcaataaagggcagtggcgtgactttgtattaaaaggacataaagatactaatcgccgtattgattacagttacgaaatcaatcccgtgggaacgccgcaggaatgtattgacataattcaaaccgacattgatgctacaggaatatcaaatatttgttgtggatttaaggctaatggaacagtagacgaaattattgcttccatgaagctcttccagtctgatgtcatgccatttcttaaagaaaaacaacgttcgctattatattgaggatcggttgtcgagtaaggatctccaggcatcaaataaaacg

SEQ ID NO: 73 - DNA, 1172 bp, Artificial Sequence
  reconstructed sequence
caattttcgtactgaaacatcttaatcatgcacaggagactttctaatgaaatttggaaactttttgcttacataccaacctccccaattttctcaaacagaggtaatgcaacgtttggttgaattaggtcgcgtgtctgaggagtgtggttttgataccgtatggttactggagcatcatttcacggagtttggtttgggtggtaacgtacaggtcgctgctgcatttttacttggcgcgactaaaaaattgaatgtaggaactgccgctattgttcttcccacagcccatccagtacgccaacttgaagatgtgaatttattggatcaaatgtcaaaaggacgatttcggtttggtatttgccgagggctttacaacaaggactttcgcgtattcggcgttgatatgaataacagtcgcgccttaatggaaaagtggtacgagcgtataaagcgtggcattacagagggatatatggaagctgataatgaacatatcaagttccataaggtaaaagtaaaccccaccgcgtatagccagggtggcgcaccgatttatgtggtggctacttcagcttcgacgactgagtgggctgctcaacatggcctaccgatgatattaagttggattataaatcgcaacgaaaagatcgcacaaattgagctttataatgaagtggctcaagaatccgggcacgatattcataatatcgaccattgcttatcatatataacatctgtagatcatgactcaattaaagcgaaagagatttgccggaactttctggggcattggtatgattcttatgtgaatgctacgactatttttgatgattcagacaagacaaaaggttatggcttcaataaagggcagtgggctgactttgtattaaaaggacataaaaatactaatcgccgtattgattacagttacgaaatcaatcccgtgggaacgccgaaggaatgtattgacataattcaaaccgacattgatgctacaggaatatcaaatatttgttgtggatttgaagctaatggaacagtagacgaaattattgcttccatgaagctcttccagaaagatgtcatgccatttcttaaagaaacgcaacgttcgctattattctgaggatcggttgtcgagtaaggatctccaggcatcaaataaaacg

SEQ ID NO: 74 - DNA, 1172 bp, Artificial Sequence
  reconstructed sequence
caattttcgtactgaaacatcttaatcatgcacaggagactttctaatgaaatttggaaactttttgcttacataccaacctccccaattttctcaaggtgaggtaatgaaacgtttggttaacttaggtcgcgtgtctgaggagtgtggttttgataccgtatggttactggagcatcatttcacggagtttggtttgcttggtaacccttatgtcgctgctgcatatttacttggcgcgactaaaaaattgaatgtaggaactgccgctattgttcttcccacagcccatccagtacgccaacttgaagatgtgaatttattggatcaaatgtcaaaaggacgatttcggtttggtatttgccgagggctttacaacaaggactttcgcgtattcggcgttgatatggataacacacgcgccttaatggaatgctggtacgggctgataaaggaaggcatgacagagggatatgtggaagctgataatgaacatatcaagttccataaggtaaaagtaaaccccaccgcgtatagcaagggtggcgcaccggtttatgtggtggctgaatcagcttcgacgactgagtgggctgctcaacatggcctaccgatgatattaagttggattataaatactaacgaaaagaaagcacaacttgattactataatgaagtggctcaagaatatgggcacgatgttcataatatcgaccattgcttatcatatataacatctgtagatcatgactcaattaaagcgaaagagatttgccggaaatttctggggcattggtatgattcttatgtgaatgctacgactatttttgatgattcagaccaaacaaaaggttatgatttcaataaagggcagtggcgtgactttgtattaaaaggacataaagatactaatcgccgtattgattacagttacgaaatcaatcccgtgggaacgccggaagaatgtattgacataattcaaaccgacattgatgctacaggaatatcaaatatttgttgtggatttgaagctaatggaacagtagacgaaattattgcttccatgaagctcttccagtctgatgtcatgccatttcttaaagaaaaacaacgttcgctattatattgaggatcggttgtcgagtaaggatctccaggcatcaaataaaacg

SEQ ID NO: 75 - DNA, 1172 bp, Artificial Sequence
  reconstructed sequence
caattttcgtactgaaacatcttaatcatgcacaggagactttctaatgaaatttggaaactttttgcttacataccaacctccccaattttctcaaacagaggtaatgcaacgtttggttaaattaggtcgcgtgtctgaggagtgtggttttgataccgtatggttactggagcatcatttcacggagtttggtttgcttggtaacccttatgtcgctgctgcatatttacttggcgcgactaaaaaattgaatgtaggaactgccgctattgttcttcccacagcccatccagtacgccaacttgaagatgtgaatttattggatcaaatgtcaaaaggacgatttcggtttggtatttgccgagggctttacaacaaggactttcgcgtattcggcacagatatggataacagtcgcgccttaatggaatgctggtacgggctgataaagaatggcatgacagagggatatgtggaagctgataatgaacatatcaagttccataaggtaaaagtaaaccccaccgcgtatagccagggtggcgcaccggtttatgtggtggctgaatcagcttcgacgactgagtgggctgctcaacatggcctaccgatgatattaagttggattataaatactaacgaaaagaaagcacaacttgagctttataatgaagtggctcaagaatatgggcacgatattcataatatcgaccattgcttatcatatataacatctgtagatcatgactcaattaaagcgaaagagatttgccggaactttctggggcattggtatgattcttatgtgaatgctacgactatttttgatgattcagaccaaacaaaaggttatgatttcaataaagggcagtggcgtgactttgtattaaaaggacataaagatactaatcgccgtattgattacagttacgaaatcaatcccgtgggaacgccgcaggaatgtattgacataattcaaaccgacattgatgctacaggaatatcaaatatttgttgtggatttgaagctaatggaacagtagacgaaattattgcttccatgaagctcttccagtctgatgtcatgccatttcttaaagaaaaacaacgttcgctattatattgaggatcggttgtcgagtaaggatctccaggcatcaaataaaacg

SEQ ID NO: 76 - DNA, 3276 bp, Artificial Sequence
  Plasmid
tcagataaaatatttctagatttcagtgcaatttatctcttcaaatgtagcacctgaagtcagccccatacgatataagttgttactagtgcttggattctcaccaataaaaaacgcccggcggcaaccgagcgttctgaacaaatccagatggagttctgaggtcattactggatctatcaacaggagtccaagcgagctcgatatcaaattacgccccgccctgccactcatcgcagtactgttgtaattcattaagcattctgccgacatggaagccatcacagacggcatgatgaacctgaatcgccagcggcatcagcaccttgtcgccttgcgtataatatttgcccatggtgaaaacgggggcgaagaagttgtccatattggccacgtttaaatcaaaactggtgaaactcacccagggattggctgagacgaaaaacatattctcaataaaccctttagggaaataggccaggttttcaccgtaacacgccacatcttgcgaatatatgtgtagaaactgccggaaatcgtcgtggtattcactccagagcgatgaaaacgtttcagtttgctcatggaaaacggtgtaacaagggtgaacactatcccatatcaccagctcaccgtctttcattgccatacggaattccggatgagcattcatcaggcgggcaagaatgtgaataaaggccggataaaacttgtgcttatttttctttacggtctttaaaaaggccgtaatatccagctgaacggtctggttataggtacattgagcaactgactgaaatgcctcaaaatgttctttacgatgccattgggatatatcaacggtggtatatccagtgatttttttctccattttagcttccttagctcctgaaaatctcgataactcaaaaaatacgcccggtagtgatcttatttcattatggtgaaagttggaacctcttacgtgccgatcaacgtctcattttcgccagatatcgacgtcgacgtcgaattcaaaagatcttaagtaagtaagagtatacgtatatcggctaataacgtattaaggcgcttcggcgcctttttttatgggggtattttcatcccaatccacacgtccaacgcacagcaaacaccacgtcgaccctatcagctgcgtgctttctatgagtcgttgctgcataacttgacaattaatcatccggctcgtataatgtgtggagggcccaagttcacttaaaaaggagatcaacaatgaaagcaattttcgtactgaaacatcttaatcatgcacaggagactttctaatgaaatttggaaactttttgcttacataccaacctccccaattttctcaaacagaggtaatgaaacgtttggttaaattaggtcgcatctctgaggagtgtggttttgataccgtatggttactggagcatcatttcacggagtttggtttgcttggtaacccttatgtcgctgctgcatatttacttggcgcgactaaaaaattgaatgtaggaactgccgctattgttcttcccacagcccatccagtacgccaacttgaagatgtgaatttattggatcaaatgtcaaaaggacgatttcggtttggtatttgccgagggctttacaacaaggactttcgcgtattcggcacagatatgaataacagtcgcgccttagcggaatgctggtacgggctgataaagaatggcatgacagagggatatatggaagctgataatgaacatatcaagttccataaggtaaaagtaaaccccgcggcgtatagcagaggtggcgcaccggtttatgtggtggctgaatcagcttcgacgactgagtgggctgctcaatttggcctaccgatgatattaagttggattataaatactaacgaaaagaaagcacaacttgagctttataatgaagtggctcaagaatatgggcacgatattcataatatcgaccattgcttatcatatataacatctgtagatcatgactcaattaaagcgaaagagatttgccggaaatttctggggcattggtatgattcttatgtgaatgctacgactatttttgatgattcagaccaaacaagaggttatgatttcaataaagggcagtggcgtgactttgtattaaaaggacataaagatactaatcgccgtattgattacagttacgaaatcaatcccgtgggaacgccgcaggaatgtattgacataattcaaaaagacattgatgctacaggaatatcaaatatttgttgtggatttgaagctaatggaacagtagacgaaattattgcttccatgaagctcttccagtctgatgtcatgccatttcttaaagaaaaacaacgttcgctattatattagggatcggttgtcgagtaaggatctccaggcatcaaataaaacgaaaggctcagtcgaaagactgggcctttcgttttatctgttgtttgtcggtgaacgctctctactagagtcacactggctcaccttcgggtgggcctttctgcgtttataggatcctaactcgagcctagggatatattccgcttcctcgctcactgactcgctacgctcggtcgttcgactgcggcgagcggaaatggcttacgaacggggcggagatttcctggaagatgccaggaagatacttaacagggaagtgagagggccgcggcaaagccgtttttccataggctccgcccccctgacaagcatcacgaaatctgacgctcaaatcagtggtggcgaaacccgacaggactataaagataccaggcgtttccccctggcggctccctcgtgcgctctcctgttcctgcctttcggtttaccggtgtcattccgctgttatggccgcgtttgtctcattccacgcctgacactcagttccgggtaggcagttcgctccaagctggactgtatgcacgaaccccccgttcagtccgaccgctgcgccttatccggtaactatcgtcttgagtccaacccggaaagacatgcaaaagcaccactggcagcagccactggtaattgatttagaggagttagtcttgaagtcatgcgccggttaaggctaaactgaaaggacaagttttggtgactgcgctcctccaagccagttacctcggttcaaagagttggtagctcagagaaccttcgaaaaaccgccctgcaaggcggttttttcgttttcagagcaagagattacgcgcagaccaaaacgatctcaagaagatcatcttattaa

SEQ ID NO: 77 - DNA, 11609 bp, Artificial Sequence
  Plasmid
tcatttcgaaccccagagtcccgctcagaagaactcgtcaagaaggcgatagaaggcgatgcgctgcgaatcgggagcggcgataccgtaaagcacgaggaagcggtcagcccattcgccgccaagctcttcagcaatatcacgggtagccaacgctatgtcctgatagcggtccgccacacccagccggccacagtcgatgaatccagaaaagcggccattttccaccatgatattcggcaagcaggcatcgccatgggtcacgacgagatcctcgccgtcgggcatgcgcgccttgagcctggcgaacagttcggctggcgcgagcccctgatgctcttcgtccagatcatcctgatcgacaagaccggcttccatccgagtacgtgctcgctcgatgcgatgtttcgcttggtggtcgaatgggcaggtagccggatcaagcgtatgcagccgccgcattgcatcagccatgatggatactttctcggcaggagcaaggtgagatgacaggagatcctgccccggcacttcgcccaatagcagccagtcccttcccgcttcagtgacaacgtcgagcacagctgcgcaaggaacgcccgtcgtggccagccacgatagccgcgctgcctcgtcctgcagttcattcagggcaccggacaggtcggtcttgacaaaaagaaccgggcgcccctgcgctgacagccggaacacggcggcatcagagcagccgattgtctgttgtgcccagtcatagccgaatagcctctccacccaagcggccggagaacctgcgtgcaatccatcttgttcaatcatgcgaaacgatcctcatcctgtctcttgatcagatcttgatcccctgcgccatcagatccttggcggcaagaaagccatccagtttactttgcagggcttcccaaccttaccagagggcgccccagccgtggcaattccggttcgctgctagacaacatcagcaaggagaaaggggctaccggcgaaccagcagcccctttataaaggcgcttcagtagtcagaccagcatcagtcctgaaaaggcgggcctgcgcccgcctccaggttgctacttaccggattcgtaagccatgaaagccgccacctccctgtgtccgtctctgtaacgaatctcgcacagcgattttcgtgtcagataagtgaatatcaacagtgtgagacacacgatcaacacacaccagacaagggaacttcgtggtagtttcatggccttcttctccttgcgcaaagcgcggtaagaggctatcctgatgtggactagacatagggatgcctcgtggtggttaatgaaaattaacttactacggggctatcttctttctgccacacaacacggcaacaaaccaccttcacgtcatgaggcagaaagcctcaagcgccgggcacatcatagcccatatacctgcacgctgaccacactcactttccctgaaaataatccgctcattcagaccgttcacgggaaatccgtgtgattgttgccgcatcacgctgcctcccggagtttgtctcgagcacttttgttacccgccaaacaaaacccaaaaacaacccatacccaacccaataaaacaccaaaacaagacaaataatcattgattgatggttgaaatggggtaaacttgacaaacaaacccacttaaaacccaaaacatacccaaacacacaccaaaaaaacaccataaggagttttataaatgttggtattcattgatgacggttcaacaaacatcaaactacagtggcaggaaagcgacggaacaattaaacagcacattagcccgaacagcttcaaacgcgagtgggcagtctcttttggtgataaaaaggtctttaactacacactgaacggcgaacagtattcatttgatccaatcagcccggatgctgtagtcacaaccaatatcgcatggcaatacagcgacgttaatgtcgttgcagtgcatcacgccttactgaccagtggtctgccggtaagcgaagtggatattgtttgcacacttcctctgacagagtattacgacagaaataaccaacccaatacggaaaatattgagcgtaagaaagcaaacttccggaaaaaaattacattaaatggcggggatacattcacaataaaagatgtaaaagtcatgcctgaatctataccggcaggttatgaagttctacaagaactggatgagttagattctttattaattatagatctcgggggcaccacattagatatttctcaggtaatggggaaattatcggggatcagtaaaatatacggagactcatctcttggtgtctctctggttacatctgcagtaaaagatgccctttctcttgcgagaacaaaaggaagtagctatcttgctgacgatataatcattcacagaaaagataataactatctgaagcaacgaattaatgatgagaacaaaatatcaatagtcaccgaagcaatgaatgaagcacttcgtaaacttgagcaacgtgtattaaatacgctcaatgaattttctggttatactcatgttatggttataggcggtggcgcagaattaatatgcgatgcagtaaaaaaacacacacagattcgtgatgaacgttttttcaaaaccaataactctcaatatgatttagttaacggtatgtatctcataggtaattaatgatggacaagcgcagaaccattgccttcaaactaaatccagatgtaaatcaaacagataaaattgtttgtgatacactggacagtatcccgcaaggggaacgaagccgccttaaccgggccgcactgacggcaggtctggccttatacagacaagatccccggacccctttccttttatgtgagctgctgacgaaagaaaccacattttcagatatcgtgaatatattgagatcgctatttccaaaagagatggccgattttaattcttcaatagtcactcaatcctcttcacaacaagagcaaaaaagtgatgaagagaccaaaaaaaatgcgatgaagctaataaattaattcaattattattgagttccctttatccactatcaggctggataaagggaactcaatcaagttattttcttaccagtcattacataatcgttattatgaaataatcgtttgcactgtctctgttattcaggcaatttcaataaaggcacttgctcacgctctgtcattttctgaaactcttcatgctggaattgataaaacagaatttgcctggcggcagtagcgcggtggtcccacctgaccccatgccgaactcagaagtgaaacgccgtagcgccgatggtagtgtggggtctccccatgcgagagtagggaactgccaggcatcaaataaaacgaaaggctcagtcgaaagactgggcctttcgttttatctgttgtttgtcggtgaacgctctcctgagtaggacaaatccgccgggagcggatttgaacgttgcgaagcaacggcccggagggtggcgggcaggacgcccgccataaactgccaggcatcaaattaagcagaaggccatcctgacggatggcctttttgcgtttctacaaactcgaattcataagaatgcggccgctgtggtagcacagaataatgaaaagtgtgtaaagaagggtaaaaaaaaccgaatgcgaggcatccggttgaaataggggtaaacagacattcagaaatgaatgacggtaataaataaagttaatgatgatagcgggagttattctagttgcgagtgaaggttttgttttgacattcagtgctgtcaaatacttaagaataagttattgattttaaccttgaattattattgcttgatgttaggtgcttatttcgccattccgcaataatcttaaaaagttcccttgcatttacattttgaaacatctatagcgataaatgaaacatcttaaaagttttagtatcatattcgtgttggattattctgcatttttggggagaatggacttgccgactgattaatgagggttaatcagtatgcagtggcataaaaaagcaaataaaggcatataacagatcgatcttaaacatccacaggaggatgggatccaaaataaggaggaaaaaaaaatgactagtatgactaaaaaaatttcattcattattaacggccaggttgaaatctttcccgaaggtgatgatttagtgcaatccattaattttggtgataatagtgtttacctgccaatattgaatgactctcatgtaaaaaacattattgattgtaatggaaataacgaattacggttgcataacattgtcaattttctctatacggtagggcaaagatggaaaaatgaagaatactcaagacgcaggacatacattcgtgacttaaaaaaatatatgggatattcagaagaaatggctaagctagaggccaattggatatctatgattttatgttctaaaggcggcctttatgatgttgtagaaaatgaacttggttctcgccatatcatggatgaatggctacctcaggatgaaagttatgttcgggcttttccgaaaggtaaatctgtacatctgttggcaggtaatgttccattatctgggatcatgtctatattacgcgcaattttaactaagaatcagtgtattataaaaacatcgtcaaccgatccttttaccgctaatgcattagcgttaagttttattgatgtagaccctaatcatccgataacgcgctctttatctgttatatattggccccaccaaggtgatacatcactcgcaaaagaaattatgcaacatgcggatgttattgtcgcttggggagggccagatgcgattaattgggcggtagagcatgcgccatcttatgctgatgtgattaaatttggttctaaaaagagtctttgcattatcgataatcctgttgatttgacgtccgcagcgacaggtgcggctcatgatgtttgtttttacgatcagcgagcttgtttttctgcccaaaacatatattacatgggaaatcattatgaggaatttaagttagcgttgatagaaaaacttaatctatatgcgcatatattaccgaatgccaaaaaagattttgatgaaaaggcggcctattctttagttcaaaaagaaagcttgtttgctggattaaaagtagaggtggatattcatcaacgttggatgattattgagtcaaatgcaggtgtggaatttaatcaaccacttggcagatgtgtgtaccttcatcacgtcgataatattgagcaaatattgccttatgttcaaaaaaataagacgcaaaccatatctatttttccttgggagtcatcatttaaatatcgagatgcgttagcattaaaaggtgcggaaaggattgtagaagcaggaatgaataacatatttcgagttggtggatctcatgacggaatgagaccgttgcaacgattagtgacatatatttctcatgaaaggccatctaactatacggctaaggatgttgcggttgaaatagaacagactcgattcctggaagaagataagttccttgtatttgtcccataataggtaaaaagtatggaaaatgaatcaaaatataaaaccatcgaccacgttatttgtgttgaaggaaataaaaaaattcatgtttgggaaacgctgccagaagaaaacagcccaaagagaaagaatgccattattattgcgtctggttttgcccgcaggatggatcattttgctggtctggcggaatatttatcgcggaatggatttcatgtgatccgctatgattcgcttcaccacgttggattgagttcagggacaattgatgaatttacaatgtctataggaaagcagagcttgttagcagtggttgattggttaactacacgaaaaataaataacttcggtatgttggcttcaagcttatctgcgcggatagcttatgcaagcctatctgaaatcaatgcttcgtttttaatcaccgcagtcggtgttgttaacttaagatattctcttgaaagagctttagggtttgattatctcagtctacccattaatgaattgccgaataatctagattttgaaggccataaattgggtgctgaagtctttgcgagagattgtcttgattttggttgggaagatttagcttctacaattaataacatgatgtatcttgatataccgtttattgcttttactgcaaataacgataattgggtcaagcaagatgaagttatcacattgttatcaaatattcgtagtaatcgatgcaagatatattctttgttaggaagttcgcatgacttgagtgaaaatttagtggtcctgcgcaatttttatcaatcggttacgaaagccgctatcgcgatggataatgatcatctggatattgatgttgatattactgaaccgtcatttgaacatttaactattgcgacagtcaatgaacgccgaatgagaattgagattgaaaatcaagcaatttctctgtcttaaaatctattgagatattctatcactcaaatagcaatataaggactctctatgaaatttggaaactttagtactcaacgttcgctattatattagctaaggagaaagaaatgaaatttggattgttcttccttaacttcatcaattcaacaactgttcaagaacaaagtatagttcgcatgcaggaaataacggagtatgttgataagttgaattttgaacagattttagtgtatgaaaatcatttttcagataatggtgttgtcggcgctcctctgactgtttctggttttctgctcggtttaacagagaaaattaaaattggttcattaaatcacatcattacaactcatcatcctgtccgcatagcggaggaagcttgcttattggatcagttaagtgaagggagatttattttagggtttagtgattgcgaaaaaaaagatgaaatgcatttttttaatcgcccggttgaatatcaacagcaactatttgaagagtgttatgaaatcattaacgatgctttaacaacaggctattgtaatccagataacgatttttatagcttccctaaaatatctgtaaatccccatgcttatacgccaggcggacctcggaaatatgtaacagcaaccagtcatcatattgttgagtgggcggccaaaaaaggtattcctctcatctttaagtgggatgattctaatgatgttagatatgaatatgctgaaagatataaagccgttgcggataaatatgacgttgacctatcagagatagaccatcagttaatgatattagttaactataacgaagatagtaataaagctaaacaagagacgcgtgcatttattagtgattatgttcttgaaatgcaccctaatgaaaatttcgaaaataaacttgaagaaataattgcagaaaacgctgtcggaaattatacggagtgtataactgcggctaagttggcaattgaaaagtgtggtgcgaaaagtgtattgctgtcctttgaaccaatgaatgatttgatgagccaaaaaaatgtaatcaatattgttgatgataatattaagaagtaccacatggaatatacctaatagatttcgagttgcagcgaggcggcaagtgaacgaatccccaggagcatagataactatgtgactggggtgagtgaaagcagccaacaaagcagcagcttgaaagatgaagggtataaaagagtatgacagcagtgctgccatactttctaatattatcttgaggagtaaaacaggtatgacttcatatgttgataaacaagaaattacagcaagctcagaaattgatgatttgattttttcgagcgatccattagtgtggtcttacgacgagcaggaaaaaatcagaaagaaacttgtgcttgatgcatttcgtaatcattataaacattgtcgagaatatcgtcactactgtcaggcacacaaagtagatgacaatattacggaaattgatgacatacctgtattcccaacatcggtttttaagtttactcgcttattaacttctcaggaaaacgagattgaaagttggtttaccagtagcggcacgaatggtttaaaaagtcaggtggcgcgtgacagattaagtattgagagactcttaggctctgtgagttatggcatgaaatatgttggtagttggtttgatcatcaaatagaattagtcaatttgggaccagatagatttaatgctcataatatttggtttaaatatgttatgagtttggtggaattgttatatcctacgacatttaccgtaacagaagaacgaatagattttgttaaaacattgaatagtcttgaacgaataaaaaatcaagggaaagatctttgtcttattggttcgccatactttatttatttactctgccattatatgaaagataaaaaaatctcattttctggagataaaagcctttatatcataaccggaggcggctggaaaagttacgaaaaagaatctctgaaacgtgatgatttcaatcatcttttatttgatactttcaatctcagtgatattagtcagatccgagatatatttaatcaagttgaactcaacacttgtttctttgaggatgaaatgcagcgtaaacatgttccgccgtgggtatatgcgcgagcgcttgatcctgaaacgttgaaacctgtacctgatggaacgccggggttgatgagttatatggatgcgtcagcaaccagttatccagcatttattgttaccgatgatgtcgggataattagcagagaatatggtaagtatcccggcgtgctcgttgaaattttacgtcgcgtcaatacgaggacgcagaaagggtgtgctttaagcttaaccgaagcgtttgatagttgatgacctgcaggcatgcaagcttgcggccgcgggccccatggatcgatagctggtcgacacaatctgccctttcgaaagatcccaacgaaaagcgtgaccacatggtccttcttgagtttgtaactgctgctgggattacacatggcatggatgagctctacaaataatgagctagctgaaaacctagcccgcctaatgagcgggcttttttttctcggcctaggtttcacctgttctattaggtgttacatgctgttcatctgttacattgtcgatctgttcatggtgaacagctttaaatgcaccaaaaactcgtaaaagctctgatgtatctatcttttttacaccgttttcatctgtgcatatggacagttttccctttgatatctaacggtgaacagttgttctacttttgtttgttagtcttgatgcttcactgatagatacaagagccataagaacctcagatccttccgtatttagccagtatgttctctagtgtggttcgttgtttttgcgtgagccatgagaacgaaccattgagatcatgcttactttgcatgtcactcaaaaattttgcctcaaaactggtgagctgaatttttgcagttaaagcatcgtgtagtgtttttcttagtccgttacgtaggtaggaatctgatgtaatggttgttggtattttgtcaccattcatttttatctggttgttctcaagttcggttacgagatccatttgtctatctagttcaacttggaaaatcaacgtatcagtcgggcggcctcgcttatcaaccaccaatttcatattgctgtaagtgtttaaatctttacttattggtttcaaaacccattggttaagccttttaaactcatggtagttattttcaagcattaacatgaacttaaattcatcaaggctaatctctatatttgccttgtgagttttcttttgtgttagttcttttaataaccactcataaatcctcatagagtatttgttttcaaaagacttaacatgttccagattatattttatgaatttttttaactggaaaagataaggcaatatctcttcactaaaaactaattctaatttttcgcttgagaacttggcatagtttgtccactggaaaatctcaaagcctttaaccaaaggattcctgatttccacagttctcgtcatcagctctctggttgctttagctaatacaccataagcattttccctactgatgttcatcatctgagcgtattggttataagtgaacgataccgtccgttctttccttgtagggttttcaatcgtggggttgagtagtgccacacagcataaaattagcttggtttcatgctccgttaagtcatagcgactaatcgctagttcatttgctttgaaaacaactaattcagacatacatctcaattggtctaggtgattttaatcactataccaattgagatgggctagtcaatgataattactagtccttttcctttgagttgtgggtatctgtaaattctgctagacctttgctggaaaacttgtaaattctgctagaccctctgtaaattccgctagacctttgtgtgttttttttgtttatattcaagtggttataatttatagaataaagaaagaataaaaaaagataaaaagaatagatcccagccctgtgtataactcactactttagtcagttccgcagtattacaaaaggatgtcgcaaacgctgtttgctcctctacaaaacagaccttaaaaccctaaaggcttaagtagcaccctcgcaagctcgggcaaatcgctgaatattccttttgtctccgaccatcaggcacctgagtcgctgtctttttcgtgacattcagttcgctgcgctcacggctctggcagtgaatgggggtaaatggcactacaggcgccttttatggattcatgcaaggaaactacccataatacaagaaaagcccgtcacgggcttctcagggcgttttatggcgggtctgctatgtggtgctatctgactttttgctgttcagcagttcctgccctctgattttccagtctgaccacttcggattatcccgtgacaggtcattcagactggctaatgcacccagtaaggcagcggtatcatcaacaggcttacccgtcttactgtcaaccggatctaaaacactaggcccaagagtttgtagaaacgcaaaaaggccatccgtcaggatggccttctgcttaatttgatgcctggcagtttatggcgggcgtcctgcccgccaccctccgggccgttgcttcgcaacgttcaaatccgctcccggcggatttgtcctactcaggagagcgttcaccgacaaacaacagataaaacgaaaggcccagtctttcgactgagcctttcgttttatttgatgcctggcagttccctactctcgcatggggagaccccacactaccatcggcgctacggcgtttcacttctgagttcggcatggggtcaggtgggaccaccgcgctactgccgccaggcaaattctgttttatcagaccgcttctgcgttctgatttaatctgtatcaggctgaaaatcttctctcatccgccaaaacagccaagctggatctaaaacactagcccaacctttcatagaaggcggcggtggaatcgaaatctcgtgatggcaggttgggcgtcgcttggtcgg